European Patent Application EP 4 137 147 A2, published February 22, 2023. Title: USES OF A PTHrP ANALOGUE IN REDUCING FRACTURE RISK. Applicant: RADIUS HEALTH, INC. The sequence listing filed with the application follows.

SEQUENCE LISTING (2 sequences)

SEQ ID NO: 1 - protein, 36 aa, Artificial Sequence
  PTHrP analogue
AVSEHQLLHDKGKSIQDLRRRELLEKLLAIBKLHTA

SEQ ID NO: 2 - protein, 34 aa, Artificial Sequence
  native hPTHrP(1-34)
AVSEHQLLHDKGKSIQDLRRRFFLHHLIAEIHTA